European Patent Specification EP 3 423 577 B1, published May 8, 2024. Title: CELLOBIOHYDROLASE VARIANTS AND POLYNUCLEOTIDES ENCODING SAME. Applicant: Novozymes A/S Wogulis, Mark DeMars, Leslie Jones, Aubrey Ding, Hanshu Osborn, David. The sequence listing filed with the application follows.

SEQUENCE LISTING (37 sequences)

SEQ ID NO: 1 - protein, 446 aa, Talaromyces leycettanus
QQTMWGQCGGQGWTGPTICVAGATCSTQNPWYAQCTPAPTAPTTLQTTTTTSSKSSTTTSSKSSTTTGGSGGGTTTSTSATITAAPSGNPYSGYQLYVNQEYSSEVYASAIPSLTGTLVAKASAAAEVPSFLWLDTASKVPLMGTYLQDIQAKNAAGANPPYAGQFVVYDLPDRDCAALASNGEYSIANNGVANYKAYIDSIRALLVQYSNVHVILVIEPDSLANLVTNLNVQKCANAQSAYLECINYALTQLNLKNVAMYIDAGHAGWLGWPANLSPAAQLFASVYQNASSPAAVRGLATNVANYNAWSIATCPSYTQGDPNCDEQKYINALAPLLQQQGWSSVHFITDTGRNGVQPTKQNAWGDWCNVIGTGFGVRPTTNTGDPLEDAFVWVKPGGESDGTSNSTSPRYDAHCGYSDALQPAPEAGTWFEAYFEQLLTNANPSF

SEQ ID NO: 2 - protein, 453 aa, Trichoderma reesei
VPLEERQACSSVWGQCGGQNWSGPTCCASGSTCVYSNDYYSQCLPGAASSSSSTRAASTTSRVSPTTSRSSSATPPPGSTTTRVPPVGSGTATYSGNPFVGVTPWANAYYASEVSSLAIPSLTGAMATAAAAVAKVPSFMWLDTLDKTPLMEQTLADIRTANKNGGNYAGQFVVYDLPDRDCAALASNGEYSIADGGVAKYKNYIDTIRQIVVEYSDIRTLLVIEPDSLANLVTNLGTPKCANAQSAYLECINYAVTQLNLPNVAMYLDAGHAGWLGWPANQDPAAQLFANVYKNASSPRALRGLATNVANYNGWNITSPPSYTQGNAVYNEKLYIHAIGPLLANHGWSNAFFITDQGRSGKQPTGQQQWGDWCNVIGTGFGIRPSANTGDSLLDSFVWVKPGGECDGTSDSSAPRFDSHCALPDALQPAPQAGAWFQAYFVQLLTNANPSFL

SEQ ID NO: 3 - protein, 450 aa, Fusarium solani
APLVEERQACAAQWAQCGGFSWNGATCCQSGSYCSKINDYYSQCIPGEGPATSKSSTLPASTTTTQPTSTSTAGTSSTTKPPPAGSGTATYSGNPYSGVNLWANSYYRSEVTNLAIPKLSGAMATAAAKVADVPSYQWMDSFDHISLMEDTLVDIRKANLAGGNYAGQFVVYDLPDRDCAAAASNGEYSLDNDGANKYKNYIQTIKKIIQSYSDIRILLVIEPDSLANLVTNMDVAKCAKAHDAYISLTNYAVTELNLPNVAMYLDAGHAGWLGWPANQGPAAKLFASIYKDAGKPAALRGLATNVANYNAWSLSSAPPYTQGASIYDEKSFIHAMGPLLEQNGWPGAHFITDQGRSGKQPTGQIQWGDWCNSKGTGFGIRPSANTGDSLLDAFVWVKPGGESDGTSDTSATRYDYHCGASAALQPAPEAGTWFQAYFEQLLTNANPSFL

SEQ ID NO: 4 - protein, 465 aa, Myceliophthora thermophila
APVIEERQNCGAVWTQCGGNGWQGPTCCASGSTCVAQNEWYSQCLPNSQVTSSTTPSSTSTSQRSTSTSSSTTRSGSSSSSSTTPPPVSSPVTSIPGGATSTASYSGNPFSGVRLFANDYYRSEVHNLAIPSMTGTLAAKASAVAEVPSFQWLDRNVTIDTLMVQTLSQVRALNKAGANPPYAAQLVVYDLPDRDCAAAASNGEFSIANGGAANYRSYIDAIRKHIIEYSDIRIILVIEPDSMANMVTNMNVAKCSNAASTYHELTVYALKQLNLPNVAMYLDAGHAGWLGWPANIQPAAELFAGIYNDAGKPAAVRGLATNVANYNAWSIASAPSYTSPNPNYDEKHYIEAFSPLLNSAGFPARFIVDTGRNGKQPTGQQQWGDWCNVKGTGFGVRPTANTGHELVDAFVWVKPGGESDGTSDTSAARYDYHCGLSDALQPAPEAGQWFQAYFEQLLTNANPPF

SEQ ID NO: 5 - protein, 451 aa, Artificial sequence
  Synthetic construct
QNCQTVWGQCGGQGWTGATSCVAGATCSTLNPYYAQCLPATATTTTTTTTPTTTTSSTTTTSTTTTSTTTTPTTTTTTTSAPSGPTTTATASGPFSGYQLYANPYYSSEVHTLAIPSLTDGSLAPKASAVAKVPSFVWLDTAAKVPTMGTYLADIQAKNKAGANPPIAGIFVVYDLPDRDCAALASNGEYSIANNGVANYKAYIDSIRAQLKKYSDVHTILVIEPDSLANLVTNLNVAKCANAQSAYLECVNYALTQLNLPNVAMYLDAGHAGWLGWPANLGPAAQLFASVYKNAGSPAAVRGLATNVANYNAWSISSCPSYTQGDSNCDEKRYINALAPLLKAQGFSDAHFIMDTSRNGVQPTKQQAWGDWCNVIGTGFGVRPTTNTGDPLEDAFVWVKPGGESDGTSDTSAARYDAHCGYSDALQPAPEAGTWFQAYFEQLLTNANPSF

SEQ ID NO: 6 - protein, 451 aa, Artificial sequence
  Synthetic construct
QNCQTVWGQCGGQGWTGATSCVAGAACSTLNPYYAQCLPATATTTTTTTTTTTTTSSTTTTSTTTSSTTTTPTTTTTTTTAPSSVTTTATASGPFSGYQLYANPYYSSEVHTLAIPSLTDGSLAPKASAVAKVPSFVWLDTAAKVPTMGTYLADIRAKNAAGANPPIAGIFVVYDLPDRDCAALASNGEYSIANNGVANYKAYIDSIRAQLVKYSDVHTILVIEPDSLANLVTNLNVAKCANAQSAYLECINYALTQLNLPNVAMYLDAGHAGWLGWPANLSPAAQLFASVYKNAGSPAALRGLATNVANYNAWSISTCPSYTQGDSNCDEKRYINALAPLLKAQGFPDAHFIMDTSRNGVQPTKQQAWGDWCNVIGTGFGVRPTTNTGDPLQDAFVWVKPGGESDGTSDTSAARYDAHCGYSDALQPAPEAGTWFQAYFEQLLTNANPSF

SEQ ID NO: 7 - protein, 451 aa, Artificial sequence
  Synthetic construct
QACQTVWGQCGGQGWTGATSCVAGAACSTLNPYYAQCLPATATTTTTTTTTTTTTSSTTTTSTTTSSTTTTPTTTTTTTSAPSGVTTTATASGPFSGYQLYANPYYSSEVHTLAIPSLTDGSLAPKATAVAKVPSFVWLDTAAKVPTMGTYLADIRAQNAAGANPPIAGIFVVYDLPDRDCAALASNGEYSIANNGVANYKAYIDSIRAQLVKYSDVHTILVIEPDSLANLVTNLNVAKCANAQSAYLECINYALTQLNLPNVAMYLDAGHAGWLGWPANLSPAAQLFASVYKNAGSPAALRGLATNVANYNAWSISTCPSYTQGDSNCDEKRYINALAPLLKEQGFSDAHFIMDTSRNGVQPTKQQAWGDWCNVIGTGFGVRPTTNTGDALQDAFVWVKPGGESDGTSDTSAARYDAHCGYSDALQPAPEAGTWFQAYFEQLLTNANPSF

SEQ ID NO: 8 - protein, 435 aa, Aspergillus fumigatus
QQTVWGQCGGQGWSGPTSCVAGAACSTLNPYYAQCIPGATATSTTLTTTTAATTTSQTTTKPTTTGPTTSAPTVTASGNPFSGYQLYANPYYSSEVHTLAMPSLPSSLQPKASAVAEVPSFVWLDVAAKVPTMGTYLADIQAKNKAGANPPIAGIFVVYDLPDRDCAALASNGEYSIANNGVANYKAYIDAIRAQLVKYSDVHTILVIEPDSLANLVTNLNVAKCANAQSAYLECVDYALKQLNLPNVAMYLDAGHAGWLGWPANLGPAATLFAKVYTDAGSPAAVRGLATNVANYNAWSLSTCPSYTQGDPNCDEKKYINAMAPLLKEAGFDAHFIMDTSRNGVQPTKQNAWGDWCNVIGTGFGVRPSTNTGDPLQDAFVWIKPGGESDGTSNSTSPRYDAHCGYSDALQPAPEAGTWFQAYFEQLLTNANPSF

SEQ ID NO: 9 - protein, 449 aa, Artificial sequence
  Synthetic construct
QAQQTVWGQCGGQGWSGPTSCVAGSTCSTQNPYYAQCIPGSTATSTTTTSTTTTTTTSTTTTTTTTTTPPTTGPTTTAPPAATTTASASGNPFSGYQLYANPYYASEVHSLAIPSLTDSSLAPKASAVAKVPSFVWLDTAAKVPTMGTYLADIQAKNKAGANPPIAGIFVVYDLPDRDCAALASNGEYSIANNGVANYKAYIDSIRAQLVKYSDVHTILVIEPDSLANLVTNLNVAKCANAQSAYLECVDYALKQLNLPNVAMYLDAGHAGWLGWPANLGPAAQLFAKVYKNAGSPAAVRGLATNVANYNAWSISTCPSYTQGDPNCDEKRYINALAPLLKENGFPDAHFIMDTSRNGVQPTKQQAWGDWCNVIGTGFGVRPTTNTGDPLQDAFVWVKPGGESDGTSNTSSPRYDAHCGYSDALQPAPEAGTWFQAYFEQLLTNANPSF

SEQ ID NO: 10 - DNA, 48 bp, Artificial sequence
  Synthetic construct
cagaagtgtgctaatgctcagagtgcttacgaggagtgcatcaactat

SEQ ID NO: 11 - DNA, 30 bp, Artificial sequence
  Synthetic construct
gtaagcactctgagcattagcacacttctg

SEQ ID NO: 12 - DNA, 48 bp, Artificial sequence
  Synthetic construct
cttagcccggccgctcaactctttgcttccgcctaccagaatgcaagc

SEQ ID NO: 13 - DNA, 30 bp, Artificial sequence
  Synthetic construct
ggaagcaaagagttgagcggccgggctaag

SEQ ID NO: 14 - DNA, 48 bp, Artificial sequence
  Synthetic construct
ctggctccattgcttcagcaacagggatgggagtcagttcactttatc

SEQ ID NO: 15 - DNA, 30 bp, Artificial sequence
  Synthetic construct
ccatccctgttgctgaagcaatggagccag

SEQ ID NO: 16 - DNA, 48 bp, Artificial sequence
  Synthetic construct
cagaagtgtgctaatgctcagagtgcttacaaggagtgcatcaactat

SEQ ID NO: 17 - DNA, 30 bp, Artificial sequence; identical to SEQ ID NO: 11
  Synthetic construct

SEQ ID NO: 18 - DNA, 48 bp, Artificial sequence
  Synthetic construct
cttagcccggccgctcaactctttgcttccgcgtaccagaatgcaagc

SEQ ID NO: 19 - DNA, 30 bp, Artificial sequence; identical to SEQ ID NO: 13
  Synthetic construct

SEQ ID NO: 20 - DNA, 48 bp, Artificial sequence
  Synthetic construct
cagaagtgtgctaatgctcagagtgcttacgtggagtgcatcaactat

SEQ ID NO: 21 - DNA, 30 bp, Artificial sequence; identical to SEQ ID NO: 11
  Synthetic construct

SEQ ID NO: 22 - DNA, 40 bp, Artificial sequence
  Synthetic construct
ttgcagccaagatctctgcacagcaaaccatgtggggtca

SEQ ID NO: 23 - DNA, 40 bp, Artificial sequence
  Synthetic construct
taaatcatattaattaagctttagaaagaggggttggcgt

SEQ ID NO: 24 - DNA, 30 bp, Artificial sequence
  Synthetic construct
gctatttttctaacaaagcatcttagatta

SEQ ID NO: 25 - DNA, 30 bp, Artificial sequence
  Synthetic construct
gctgatcccctcgttttcggaaacgctttg

SEQ ID NO: 26 - DNA, 30 bp, Artificial sequence
  Synthetic construct
ggtccgttaaggttagaagaaggctacttt

SEQ ID NO: 27 - DNA, 30 bp, Artificial sequence
  Synthetic construct
cctattccgaagttcctattctctagaaag

SEQ ID NO: 28 - DNA, 30 bp, Artificial sequence
  Synthetic construct
ttgctatgtacatcgatgctggtcatgctg

SEQ ID NO: 29 - DNA, 30 bp, Artificial sequence
  Synthetic construct
cagcatgaccagcatcgatgtacatagcaa

SEQ ID NO: 30 - DNA, 30 bp, Artificial sequence
  Synthetic construct
gagcagaaatacatcaacgctctggctcca

SEQ ID NO: 31 - DNA, 30 bp, Artificial sequence
  Synthetic construct
tggagccagagcgttgatgtatttctgctc

SEQ ID NO: 32 - DNA, 500 bp, Talaromyces leycettanus
tgtaagatcaccctctgtgtattgcaccatgcggtctctcctggctcttgcccctaccctgctcgcgcctgttgttcaggctcagcaaaccatgtggggtcaatgcggtggtcagggctggaccggacctaccatctgtgtagcaggcgcgacatgcagcacacagaacccttggtatgcgcagtgcaccccagcacctaccgcgccgacgaccttgcaaacaacaactacgacgagctcgaaatcgtccacgaccacgagctcgaagtcgtccacgaccacaggtggaagtggcggtggaactacgacctcaacgtcagccaccatcaccgcggctccatctggtaacccatactccggataccagctctatgtgaaccaggaatactcgtccgaggtgtacgcgtctgctattccttcccttaccggcactctggtcgcgaaggcaagcgccgcggcagaggtgccatctttcctgtggctggacactgcctccaagg

SEQ ID NO: 33 - DNA, 500 bp, Talaromyces leycettanus
gaggtgccatctttcctgtggctggacactgcctccaaggtgccactgatgggcacttacttgcaggatatccaggcgaagaacgctgctggcgccaacccaccatatgccggtcaattcgtggtttacgacttgccggatcgtgattgcgctgcattggccagcaatggagagtactccattgctaacaatggtgttgccaactacaaggcttacatcgactccatccgcgcgcttcttgttcaatactcgaacgtccatgtcatccttgtgatcgagcccgacagcttggccaaccttgtcaccaacctgaatgttcagaagtgtgctaatgctcagagtgcttacctggagtgcatcaactatgccctcactcagttgaacctcaagaacgttgctatgtacatcgatgctggtcatgctggatggctcggctggcccgccaaccttagcccggccgctcaactctttgcttccgtataccagaatgcaagctcccc

SEQ ID NO: 34 - DNA, 500 bp, Talaromyces leycettanus
tgcttccgtataccagaatgcaagctccccagctgccgttcgcggcctggcaaccaacgtggccaactataatgcctggtcgatcgccacttgcccatcttacacccaaggcgaccccaactgcgacgagcagaaatacatcaacgctctggctccattgcttcagcaacagggatggtcatcagttcactttatcaccgataccggccgtaacggtgtccagcctaccaagcagaatgcctggggtgactggtgcaacgttatcggaaccggcttcggtgtccgtcccaccaccaacactggcgatccattggaggatgctttcgtctgggtcaagcctggtggtgagagtgatggtacttccaactccacttcgcctcgctacgacgcccactgcggttacagtgatgctcttcagcctgctcctgaggctggtacctggttcgaggcttactttgagcaactccttaccaacgccaacccctctttctaatagttaa

SEQ ID NO: 35 - DNA, 48 bp, Artificial sequence
  Synthetic constuct
gcagctcacctgaagaggcttgtaagatcaccctctgtgtattgcacc

SEQ ID NO: 36 - DNA, 49 bp, Artificial sequence
  Synthetic construct
ccaacgccaacccctctttctaatagttaattaaggctttcgtgaccgg

SEQ ID NO: 37 - DNA, 57 bp, Saccharomyces cerevisiae
atgcttttgcaagccttccttttccttttggctggttttgcagccaagatctctgca